European Patent Specification EP 4 108 782 B1, published June 7, 2023. Title: COMPOSITIONS AND METHODS FOR ANALYTE DETECTION. Applicant: PRESIDENT AND FELLOWS OF HARVARD COLLEGE. Application PCT/US12/71398. The sequence listing filed with the application follows.

SEQUENCE LISTING (82 sequences)

SEQ ID NO: 1 - DNA, 18 bp, Artificial Sequence
  Description of Artificial Sequence: Synthetic probe
cctacacaccagcgtgcc

SEQ ID NO: 2 - DNA, 18 bp, Artificial Sequence
  Description of Artificial Sequence: Synthetic probe
ccgcactttcatcttccg

SEQ ID NO: 3 - DNA, 18 bp, Artificial Sequence
  Description of Artificial Sequence: Synthetic probe
gccaaggcttatactcgc

SEQ ID NO: 4 - DNA, 18 bp, Artificial Sequence
  Description of Artificial Sequence: Synthetic probe
gctgcctcccgtaggagt

SEQ ID NO: 5 - DNA, 43 bp, Artificial Sequence
  Description of Artificial Sequence: Synthetic probe
ctgcctcccgtaggagttttttcgctttagcctaagtgaaatc

SEQ ID NO: 6 - DNA, 19 bp, Artificial Sequence
  Description of Artificial Sequence: Synthetic probe
ctctggcttcaccctattc

SEQ ID NO: 7 - DNA, 45 bp, Artificial Sequence
  Description of Artificial Sequence: Synthetic probe
ctctggcttcaccctattctttttcgcttttttggggaaaagaca

SEQ ID NO: 8 - DNA, 18 bp, Artificial Sequence
  Description of Artificial Sequence: Synthetic probe
cggaagattccctactgc

SEQ ID NO: 9 - DNA, 44 bp, Artificial Sequence
  Description of Artificial Sequence: Synthetic probe
cggaagattccctactgctttttcgctttctgtaatggagtgga

SEQ ID NO: 10 - DNA, 18 bp, Artificial Sequence
  Description of Artificial Sequence: Synthetic probe
tcctccatatctctgcgc

SEQ ID NO: 11 - DNA, 19 bp, Artificial Sequence
  Description of Artificial Sequence: Synthetic probe
gaagcaagcttctcgtccg

SEQ ID NO: 12 - DNA, 18 bp, Artificial Sequence
  Description of Artificial Sequence: Synthetic probe
cactctccccttctgcac

SEQ ID NO: 13 - DNA, 18 bp, Artificial Sequence
  Description of Artificial Sequence: Synthetic probe
gtgatgcaagtgcacctt

SEQ ID NO: 14 - DNA, 20 bp, Artificial Sequence
  Description of Artificial Sequence: Synthetic probe
ttccaaagcgtacattggtt

SEQ ID NO: 15 - DNA, 20 bp, Artificial Sequence
  Description of Artificial Sequence: Synthetic probe
gtaaacaccaaacmtcagcg

SEQ ID NO: 16 - DNA, 19 bp, Artificial Sequence
  Description of Artificial Sequence: Synthetic probe
cgaaggggacgtcctatct

SEQ ID NO: 17 - DNA, 18 bp, Artificial Sequence
  Description of Artificial Sequence: Synthetic probe
caggcttgctcctcgttg

SEQ ID NO: 18 - DNA, 18 bp, Artificial Sequence
  Description of Artificial Sequence: Synthetic probe
tctcggccttgaaacccc

SEQ ID NO: 19 - DNA, 18 bp, Artificial Sequence
  Description of Artificial Sequence: Synthetic probe
cctacacaccagcgtgcc

SEQ ID NO: 20 - DNA, 18 bp, Artificial Sequence
  Description of Artificial Sequence: Synthetic probe
ccgcactttcatcttccg

SEQ ID NO: 21 - DNA, 18 bp, Artificial Sequence
  Description of Artificial Sequence: Synthetic probe
ctgtgcgccggttctctt

SEQ ID NO: 22 - DNA, 20 bp, Artificial Sequence
  Description of Artificial Sequence: Synthetic probe
ctacaagactccagcctgcc

SEQ ID NO: 23 - DNA, 27 bp, Artificial Sequence
  Description of Artificial Sequence: Synthetic probe
atgagcaaaggtattaactttactccc

SEQ ID NO: 24 - DNA, 23 bp, Artificial Sequence
  Description of Artificial Sequence: Synthetic probe
agctaatcccacctaggttcatc

SEQ ID NO: 25 - DNA, 21 bp, Artificial Sequence
  Description of Artificial Sequence: Synthetic probe
cacacctgactgactatcccg

SEQ ID NO: 26 - DNA, 19 bp, Artificial Sequence
  Description of Artificial Sequence: Synthetic probe
gccaaggcttatactcgct

SEQ ID NO: 27 - DNA, 19 bp, Artificial Sequence
  Description of Artificial Sequence: Synthetic probe
ccgccaagccacaaggact

SEQ ID NO: 28 - DNA, 18 bp, Artificial Sequence
  Description of Artificial Sequence: Synthetic probe
gattctcggccccatggg

SEQ ID NO: 29 - DNA, 19 bp, Artificial Sequence
  Description of Artificial Sequence: Synthetic probe
cctggttcgccaaaaaggc

SEQ ID NO: 30 - DNA, 96 bp, Artificial Sequence
  Description of Artificial Sequence: Synthetic probe
tcctccatatctctgcgctttttcgctttctggagaaagggccatttttcgctttcggttccaaagacactttttcgctttctggagaaagggcca

SEQ ID NO: 31 - DNA, 97 bp, Artificial Sequence
  Description of Artificial Sequence: Synthetic probe
gaagcaagcttctcgtccgtttttcgctttctggagaaagggccatttttcgctttcggttccaaagacactttttcgctttggaagcacctattcc

SEQ ID NO: 32 - DNA, 96 bp, Artificial Sequence
  Description of Artificial Sequence: Synthetic probe
cactctccccttctgcactttttcgctttctggagaaagggccatttttcgcttttcacgatcccatgtatttttcgctttctggagaaagggcca

SEQ ID NO: 33 - DNA, 96 bp, Artificial Sequence
  Description of Artificial Sequence: Synthetic probe
gtgatgcaagtgcacctttttttcgctttgaagccggttatagctttttcgcttttaggcattagcattgtttttcgcttttcacgatcccatgta

SEQ ID NO: 34 - DNA, 98 bp, Artificial Sequence
  Description of Artificial Sequence: Synthetic probe
ttccaaagcgtacattggtttttttcgctttcggttccaaagacactttttcgctttggaagcacctattcctttttcgcttttcacgatcccatgta

SEQ ID NO: 35 - DNA, 98 bp, Artificial Sequence
  Description of Artificial Sequence: Synthetic probe
gtaaacaccaaacmtcagcgtttttcgctttgaagccggttatagctttttcgctttctggagaaagggccatttttcgcttttcacgatcccatgta

SEQ ID NO: 36 - DNA, 97 bp, Artificial Sequence
  Description of Artificial Sequence: Synthetic probe
cgaaggggacgtcctatcttttttcgcttttcacgatcccatgtatttttcgctttggaagcacctattcctttttcgcttttcacgatcccatgta

SEQ ID NO: 37 - DNA, 96 bp, Artificial Sequence
  Description of Artificial Sequence: Synthetic probe
caggcttgctcctcgttgtttttcgctttctggagaaagggccatttttcgctttgaagccggttatagctttttcgctttctggagaaagggcca

SEQ ID NO: 38 - DNA, 70 bp, Artificial Sequence
  Description of Artificial Sequence: Synthetic probe
tctcggccttgaaacccctttttcgcttttaggcattagcattgtttttcgctttcggttccaaagacac

SEQ ID NO: 39 - DNA, 96 bp, Artificial Sequence
  Description of Artificial Sequence: Synthetic probe
cctacacaccagcgtgcctttttcgcttttcacgatcccatgtatttttcgcttttaggcattagcattgtttttcgcttttcacgatcccatgta

SEQ ID NO: 40 - DNA, 96 bp, Artificial Sequence
  Description of Artificial Sequence: Synthetic probe
ccgcactttcatcttccgtttttcgctttcggttccaaagacactttttcgcttttaggcattagcattgtttttcgctttgaagccggttatagc

SEQ ID NO: 41 - DNA, 96 bp, Artificial Sequence
  Description of Artificial Sequence: Synthetic probe
ctgtgcgccggttctctttttttcgctttctggagaaagggccatttttcgctttcggttccaaagacactttttcgctttctggagaaagggcca

SEQ ID NO: 42 - DNA, 98 bp, Artificial Sequence
  Description of Artificial Sequence: Synthetic probe
ctacaagactccagcctgcctttttcgctttctggagaaagggccatttttcgctttgaagccggttatagctttttcgctttctggagaaagggcca

SEQ ID NO: 43 - DNA, 79 bp, Artificial Sequence
  Description of Artificial Sequence: Synthetic probe
atgagcaaaggtattaactttactccctttttcgcttttaggcattagcattgtttttcgctttgaagccggttatagc

SEQ ID NO: 44 - DNA, 101 bp, Artificial Sequence
  Description of Artificial Sequence: Synthetic probe
agctaatcccacctaggttcatctttttcgcttttaggcattagcattgtttttcgctttcggttccaaagacactttttcgctttggaagcacctattcc

SEQ ID NO: 45 - DNA, 73 bp, Artificial Sequence
  Description of Artificial Sequence: Synthetic probe
cacacctgactgactatcccgtttttcgctttggaagcacctattcctttttcgctttcggttccaaagacac

SEQ ID NO: 46 - DNA, 97 bp, Artificial Sequence
  Description of Artificial Sequence: Synthetic probe
gccaaggcttatactcgcttttttcgctttcggttccaaagacactttttcgctttggaagcacctattcctttttcgctttgaagccggttatagc

SEQ ID NO: 47 - DNA, 97 bp, Artificial Sequence
  Description of Artificial Sequence: Synthetic probe
ccgccaagccacaaggacttttttcgctttgaagccggttatagctttttcgctttggaagcacctattcctttttcgcttttcacgatcccatgta

SEQ ID NO: 48 - DNA, 96 bp, Artificial Sequence
  Description of Artificial Sequence: Synthetic probe
gattctcggccccatgggtttttcgcttttaggcattagcattgtttttcgctttgaagccggttatagctttttcgctttggaagcacctattcc

SEQ ID NO: 49 - DNA, 97 bp, Artificial Sequence
  Description of Artificial Sequence: Synthetic probe
cctggttcgccaaaaaggctttttcgctttctggagaaagggccatttttcgctttgaagccggttatagctttttcgctttggaagcacctattcc

SEQ ID NO: 50 - DNA, 21 bp, Artificial Sequence
  Description of Artificial Sequence: Synthetic probe
cgctttctgtaatggagtgga

SEQ ID NO: 51 - DNA, 21 bp, Artificial Sequence
  Description of Artificial Sequence: Synthetic probe
cgctttagcctaagtgaaatc

SEQ ID NO: 52 - DNA, 21 bp, Artificial Sequence
  Description of Artificial Sequence: Synthetic probe
cgcttttttggggaaaagaca

SEQ ID NO: 53 - DNA, 21 bp, Artificial Sequence
  Description of Artificial Sequence: Synthetic probe
cgcttttaggcattagcattg

SEQ ID NO: 54 - DNA, 21 bp, Artificial Sequence
  Description of Artificial Sequence: Synthetic probe
cgctttggaagcacctattcc

SEQ ID NO: 55 - DNA, 21 bp, Artificial Sequence
  Description of Artificial Sequence: Synthetic probe
cgctttctggagaaagggcca

SEQ ID NO: 56 - DNA, 21 bp, Artificial Sequence
  Description of Artificial Sequence: Synthetic probe
cgctttcggttccaaagacac

SEQ ID NO: 57 - DNA, 21 bp, Artificial Sequence
  Description of Artificial Sequence: Synthetic probe
cgctttgaagccggttatagc

SEQ ID NO: 58 - DNA, 21 bp, Artificial Sequence
  Description of Artificial Sequence: Synthetic probe
cgcttttcacgatcccatgta

SEQ ID NO: 59 - DNA, 24 bp, Artificial Sequence
  Description of Artificial Sequence: Synthetic oligonucleotide
  5'-Biotin
tttcgctttctgtaatggagtgga

SEQ ID NO: 60 - DNA, 24 bp, Artificial Sequence
  Description of Artificial Sequence: Synthetic oligonucleotide
  5'-Biotin
tttcgctttagcctaagtgaaatc

SEQ ID NO: 61 - DNA, 24 bp, Artificial Sequence
  Description of Artificial Sequence: Synthetic oligonucleotide
  5'-Biotin
tttcgcttttttggggaaaagaca

SEQ ID NO: 62 - DNA, 24 bp, Artificial Sequence
  Description of Artificial Sequence: Synthetic oligonucleotide
  5'-Biotin
tttcgcttttaggcattagcattg

SEQ ID NO: 63 - DNA, 24 bp, Artificial Sequence
  Description of Artificial Sequence: Synthetic oligonucleotide
  5'-Biotin
tttcgctttggaagcacctattcc

SEQ ID NO: 64 - DNA, 24 bp, Artificial Sequence
  Description of Artificial Sequence: Synthetic oligonucleotide
  5'-Biotin
tttcgctttctggagaaagggcca

SEQ ID NO: 65 - DNA, 24 bp, Artificial Sequence
  Description of Artificial Sequence: Synthetic oligonucleotide
  5'-Biotin
tttcgctttcggttccaaagacac

SEQ ID NO: 66 - DNA, 24 bp, Artificial Sequence
  Description of Artificial Sequence: Synthetic oligonucleotide
  5'-Biotin
tttcgctttgaagccggttatagc

SEQ ID NO: 67 - DNA, 18 bp, Artificial Sequence
  Description of Artificial Sequence: Synthetic probe
  5'-FAM
ttttccactccattacag

SEQ ID NO: 68 - DNA, 18 bp, Artificial Sequence
  Description of Artificial Sequence: Synthetic probe
  5'-Cy3
tttgatttcacttaggct

SEQ ID NO: 69 - DNA, 18 bp, Artificial Sequence
  Description of Artificial Sequence: Synthetic probe
  5'-Cy5
ttttgtcttttccccaaa

SEQ ID NO: 70 - DNA, 18 bp, Artificial Sequence
  Description of Artificial Sequence: Synthetic probe
  5'-FAM
tttcaatgctaatgccta

SEQ ID NO: 71 - DNA, 18 bp, Artificial Sequence
  Description of Artificial Sequence: Synthetic probe
  5'-Cy3
tttggaataggtgcttcc

SEQ ID NO: 72 - DNA, 18 bp, Artificial Sequence
  Description of Artificial Sequence: Synthetic probe
  5'-Cy5
ttttggccctttctccag

SEQ ID NO: 73 - DNA, 18 bp, Artificial Sequence
  Description of Artificial Sequence: Synthetic probe
  5'-FAM
tttgtgtctttggaaccg

SEQ ID NO: 74 - DNA, 18 bp, Artificial Sequence
  Description of Artificial Sequence: Synthetic probe
  5'-Cy3
tttgctataaccggcttc

SEQ ID NO: 75 - DNA, 21 bp, Artificial Sequence
  Description of Artificial Sequence: Synthetic probe
tccactccattacagaaagcg

SEQ ID NO: 76 - DNA, 21 bp, Artificial Sequence
  Description of Artificial Sequence: Synthetic probe
gatttcacttaggctaaagcg

SEQ ID NO: 77 - DNA, 21 bp, Artificial Sequence
  Description of Artificial Sequence: Synthetic probe
tgtcttttccccaaaaaagcg

SEQ ID NO: 78 - DNA, 21 bp, Artificial Sequence
  Description of Artificial Sequence: Synthetic probe
caatgctaatgcctaaaagcg

SEQ ID NO: 79 - DNA, 21 bp, Artificial Sequence
  Description of Artificial Sequence: Synthetic probe
ggaataggtgcttccaaagcg

SEQ ID NO: 80 - DNA, 21 bp, Artificial Sequence
  Description of Artificial Sequence: Synthetic probe
tggccctttctccagaaagcg

SEQ ID NO: 81 - DNA, 22 bp, Artificial Sequence
  Description of Artificial Sequence: Synthetic probe
tgtgtctttggaaccgaaagcg

SEQ ID NO: 82 - DNA, 21 bp, Artificial Sequence
  Description of Artificial Sequence: Synthetic probe
gctataaccggcttcaaagcg